European Patent Specification EP 3 341 409 B1, published February 25, 2026. Title: BIOPHARMACEUTICAL COMPOSITIONS. Applicant: GlaxoSmithKline LLC Bam, Narendra Monck, Myrna Dally, Jennifer Spatara, Michelle. The sequence listing filed with the application follows.

SEQUENCE LISTING (14 sequences)

SEQ ID NO: 1 - protein, 449 aa, Artificial Sequence
  Amino acid sequence identified using molecular biology techniques.
QVTLRESGPALVKPTQTLTLTCTVSGFSLTSYSVHWVRQPPGKGLEWLGVIWASGGTDYNSALMSRLSISKDTSRNQVVLTMTNMDPVDTATYYCARDPPSSLLRLDYWGRGTPVTVSSASTKGPSVFPLAPSSKSTSGGTAALGCLVKDYFPEPVTVSWNSGALTSGVHTFPAVLQSSGLYSLSSVVTVPSSSLGTQTYICNVNHKPSNTKVDKRVEPKSCDKTHTCPPCPAPELLGGPSVFLFPPKPKDTLMISRTPEVTCVVVDVSHEDPEVKFNWYVDGVEVHNAKTKPREEQYNSTYRVVSVLTVLHQDWLNGKEYKCKVSNKALPAPIEKTISKAKGQPREPQVYTLPPSREEMTKNQVSLTCLVKGFYPSDIAVEWESNGQPENNYKTTPPVLDSDGSFFLYSKLTVDKSRWQQGNVFSCSVMHEALHNHYTQKSLSLSPGK

SEQ ID NO: 2 - protein, 220 aa, Artificial Sequence
  Amino acid sequence identified using molecular biology techniques.
DIVMTQSPDSLAVSLGERATINCKSSQSLLNSGNQKNYLAWYQQKPGQPPKLLIYGASTRESGVPDRFSGSGSGTDFTLTISSLQAEDVAVYYCQNVHSFPFTFGGGTKLEIKRTVAAPSVFIFPPSDEQLKSGTASVVCLLNNFYPREAKVQWKVDNALQSGNSQESVTEQDSKDSTYSLSSTLTLSKADYEKHKVYACEVTHQGLSSPVTKSFNRGEC

SEQ ID NO: 3 - protein, 119 aa, Artificial Sequence [sequence omitted]

SEQ ID NO: 4 - protein, 113 aa, Artificial Sequence [sequence omitted]

SEQ ID NO: 5 - protein, 5 aa, Artificial Sequence
  Amino acid sequence identified using molecular biology techniques.
SYSVH

SEQ ID NO: 6 - protein, 16 aa, Artificial Sequence
  Amino acid sequence identified using molecular biology techniques.
VIWASGGTDYNSALMS

SEQ ID NO: 7 - protein, 11 aa, Artificial Sequence
  Amino acid sequence identified using molecular biology techniques.
DPPSSLLRLDY

SEQ ID NO: 8 - protein, 17 aa, Artificial Sequence
  Amino acid sequence identified using molecular biology techniques.
KSSQSLLNSGNQKNYLA

SEQ ID NO: 9 - protein, 7 aa, Artificial Sequence
  Amino acid sequence identified using molecular biology techniques.
GASTRES

SEQ ID NO: 10 - protein, 9 aa, Artificial Sequence
  Amino acid sequence identified using molecular biology techniques.
QNVHSFPFT

SEQ ID NO: 11 - protein, 115 aa, Artificial Sequence
  Amino acid sequence identified using molecular biology techniques.
IPTEIPTSALVKETLALLSTHRTLLIANETLRIPVPVHKNHQLCTEEIFQGIGTLESQTVQGGTVERLFKNLSLIKKYIDGQKKKCGEERRRVNQFLDYLQEFLGVMNTEWIIES

SEQ ID NO: 12 - protein, 400 aa, Artificial Sequence
  Amino acid sequence identified using molecular biology techniques.
DLLPDEKISLLPPVNFTIKVTGLAQVLLQWKPNPDQEQRNVNLEYQVKINAPKEDDYETRITESKCVTILHKGFSASVRTILQNDHSLLASSWASAELHAPPGSPGTSIVNLTCTTNTTEDNYSRLRSYQVSLHCTWLVGTDAPEDTQYFLYYRYGSWTEECQEYSKDTLGRNIACWFPRTFILSKGRDWLAVLVNGSSKHSAIRPFDQLFALHAIDQINPPLNVTAEIEGTRLSIQWEKPVSAFPIHCFDYEVKIHNTRNGYLQIEKLMTNAFISIIDDLSKYDVQVRAAVSSMCREAGLWSEWSQPIYVGNDEHKPLREWFVIVIMATICFILLILSLICKICHLWIKLFPPIPAPKSNIKDLFVTTNYEKAGSSETEIEVICYIEKPGVETLEDSVF

SEQ ID NO: 13 - DNA, 1347 bp, Artificial Sequence
  Nucleic acid sequence identified using molecular biology techniques.
caggttaccctgcgtgaatccggtccggcactagttaaaccgacccagaccctgacgttaacctgcaccgtctccggtttctccctgacgagctatagtgtacactgggtccgtcagccgccgggtaaaggtctagaatggctgggtgtaatatgggctagtggaggcacagattataattcggctctcatgtcccgtctgtcgatatccaaagacacctcccgtaaccaggttgttctgaccatgactaacatggacccggttgacaccgctacctactactgcgctcgagatcccccttcttccttactacggcttgactactggggtcgtggtaccccagttaccgtgagctcagctagtaccaagggcccatcggtcttccccctggcaccctcctccaagagcacctctgggggcacagcggccctgggctgcctggtcaaggactacttccccgaaccggtgacggtgtcgtggaactcaggcgccctgaccagcggcgtgcacaccttcccggctgtcctacagtcctcaggactctactccctcagcagcgtggtgaccgtgccctccagcagcttgggcacccagacctacatctgcaacgtgaatcacaagcccagcaacaccaaggtggacaagagagttgagcccaaatcttgtgacaaaactcacacatgcccaccgtgcccagcacctgaactcctggggggaccgtcagtcttcctcttccccccaaaacccaaggacaccctcatgatctcccggacccctgaggtcacatgcgtggtggtggacgtgagccacgaagaccctgaggtcaagttcaactggtacgtggacggcgtggaggtgcataatgccaagacaaagccgcgggaggagcagtacaacagcacgtaccgtgtggtcagcgtcctcaccgtcctgcaccaggactggctgaatggcaaggagtacaagtgcaaggtctccaacaaagccctcccagcccccatcgagaaaaccatctccaaagccaaagggcagccccgagaaccacaggtgtacaccctgcccccatcccgggaggagatgaccaagaaccaggtcagcctgacctgcctggtcaaaggcttctatcccagcgacatcgccgtggagtgggagagcaatgggcagccggagaacaactacaagaccacgcctcccgtgctggactccgacggctccttcttcctctatagcaagctcaccgtggacaagagcaggtggcagcaggggaacgtcttctcatgctccgtgatgcatgaggctctgcacaaccactacacgcagaagagcctctccctgtctccgggtaag

SEQ ID NO: 14 - DNA, 660 bp, Artificial Sequence
  Nucleic acid sequence identified using molecular biology techniques.
gatatcgtgatgacccagtctccagactcgctagctgtgtctctgggcgagagggccaccatcaactgcaagagctctcagagtctgttaaacagtggaaatcaaaagaactacttggcctggtatcagcagaaacccgggcagcctcctaagttgctcatttacggggcgtcgactagggaatctggggtacctgaccgattcagtggcagcgggtctgggacagatttcactctcaccatcagcagcctgcaggctgaagatgtggcagtatactactgtcagaatgttcatagttttccattcacgttcggcggagggaccaagttggagatcaaacgtactgtggcggcgccatctgtcttcatcttcccgccatctgatgagcagttgaaatctggaactgcctctgttgtgtgcctgctgaataacttctatcccagagaggccaaagtacagtggaaggtggataacgccctccaatcgggtaactcccaggagagtgtcacagagcaggacagcaaggacagcacctacagcctcagcagcaccctgacgctgagcaaagcagactacgagaaacacaaagtctacgcctgcgaagtcacccatcagggcctgagctcgcccgtcacaaagagcttcaacaggggagagtgt